European Patent Specification EP 3 556 869 B1, published August 2, 2023. Title: COMPOSITIONS AND METHODS FOR POLYNUCLEOTIDE SEQUENCING. Applicant: ILLUMINA, INC. The sequence listing filed with the application follows.

SEQUENCE LISTING (90 sequences)

SEQ ID NO: 1 - protein, 184 aa, Artificial Sequence
  source: /note="Description of Artificial Sequence: Synthetic polypeptide"
GLDNELSLVDGQDRTLTVQQWDTFLNGVFPLDRNRLTREWFHSGRAKYIVAGPGADEFEGTLELGYQIGFPWSLGVGINFSYTTPNILINNGNITAPPFGLNSVITPNLFPGVSISARLGNGPGIQEVATFSVRVSGAKGGVAVSNAHGTVTGAAGGVLLRPFARLIASTGDSVTTYGEPWNMN

SEQ ID NO: 2 - protein, 4 aa, Unknown
  source: /note="Description of Unknown: 'DEAD' box motif sequence"
DEAD

SEQ ID NO: 3 - protein, 4 aa, Unknown
  source: /note="Description of Unknown: 'DEAH' box motif sequence"
DEAH

SEQ ID NO: 4 - protein, 8 aa, Methanococcoides burtonii
QMAGRAGR

SEQ ID NO: 5 - protein, 9 aa, Methanococcoides burtonii
QMAGRAGRP

SEQ ID NO: 6 - protein, 8 aa, Pyrococcus furiosus
QMLGRAGR

SEQ ID NO: 7 - protein, 9 aa, Pyrococcus furiosus
QMLGRAGRP

SEQ ID NO: 8 - protein, 8 aa, Haloferax volcanii
QMMGRAGR

SEQ ID NO: 9 - protein, 9 aa, Haloferax volcanii
QMMGRAGRP

SEQ ID NO: 10 - protein, 8 aa, Halorubrum lacusprofundi
QMCGRAGR

SEQ ID NO: 11 - protein, 8 aa, Halorubrum lacusprofundi
QMGRAGRP

SEQ ID NO: 12 - protein, 8 aa, Cenarchaeum symbiosum
QLCGRAGR

SEQ ID NO: 13 - protein, 9 aa, Cenarchaeum symbiosum
QLCGRAGRP

SEQ ID NO: 14 - protein, 8 aa, Sulfolobus solfataricus
QMSGRAGR

SEQ ID NO: 15 - protein, 9 aa, Sulfolobus solfataricus
QMSGRAGRP

SEQ ID NO: 16 - protein, 8 aa, Methanogenium frigidum
QMAGRAGR

SEQ ID NO: 17 - protein, 9 aa, Methanogenium frigidum
QMAGRAGRP

SEQ ID NO: 18 - protein, 8 aa, Methanothermococcus okinawensis
QCIGRAGR

SEQ ID NO: 19 - protein, 9 aa, Methanothermococcus okinawensis
QCIGRAGRP

SEQ ID NO: 20 - protein, 8 aa, Methanotorris igneus
QCIGRAGR

SEQ ID NO: 21 - protein, 9 aa, Methanotorris igneus
QCIGRAGRP

SEQ ID NO: 22 - protein, 8 aa, Thermococcus gammatolerans
QMMGRAGR

SEQ ID NO: 23 - protein, 9 aa, Thermococcus gammatolerans
QMMGRAGRP

SEQ ID NO: 24 - protein, 8 aa, Thermococcus barophilus
QMIGRAGR

SEQ ID NO: 25 - protein, 9 aa, Thermococcus barophilus
QMIGRAGRP

SEQ ID NO: 26 - protein, 8 aa, Thermococcus sibiricus
QMMGRAGR

SEQ ID NO: 27 - protein, 9 aa, Thermococcus sibiricus
QMMGRAGRP

SEQ ID NO: 28 - protein, 8 aa, Methanosarcina barkeri
QMAGRAGR

SEQ ID NO: 29 - protein, 9 aa, Methanosarcina barkeri
QMAGRAGRP

SEQ ID NO: 30 - protein, 8 aa, Methanosarcina acetivorans
QMAGRAGR

SEQ ID NO: 31 - protein, 9 aa, Methanosarcina acetivorans
QMAGRAGRP

SEQ ID NO: 32 - protein, 8 aa, Methanohalophilus mahii
QMAGRAGR

SEQ ID NO: 33 - protein, 9 aa, Methanohalophilus mahii
QMAGRAGRP

SEQ ID NO: 34 - protein, 8 aa, Methanosarcina mazei
QMAGRAGR

SEQ ID NO: 35 - protein, 9 aa, Methanosarcina mazei
QMAGRAGRP

SEQ ID NO: 36 - protein, 8 aa, Methanosaeta thermophila
QMAGRAGR

SEQ ID NO: 37 - protein, 9 aa, Methanosaeta thermophila
QMAGRAGRP

SEQ ID NO: 38 - protein, 8 aa, Methanosalsum zhilinae
QMAGRAGR

SEQ ID NO: 39 - protein, 9 aa, Methanosalsum zhilinae
QMAGRAGRP

SEQ ID NO: 40 - protein, 8 aa, Methanohalobium evestigatum
QMAGRAGR

SEQ ID NO: 41 - protein, 9 aa, Methanohalobium evestigatum
QMAGRAGRP

SEQ ID NO: 42 - protein, 8 aa, Methanococcus maripaludis
QCIGRAGR

SEQ ID NO: 43 - protein, 9 aa, Methanococcus maripaludis
QCIGRAGRP

SEQ ID NO: 44 - protein, 8 aa, Natrialba magadii
QMMGRAGR

SEQ ID NO: 45 - protein, 9 aa, Natrialba magadii
QMMGRAGRP

SEQ ID NO: 46 - protein, 8 aa, Methanoregula boonci
QMAGRAGR

SEQ ID NO: 47 - protein, 9 aa, Methanoregula boonci
QMAGRAGRP

SEQ ID NO: 48 - protein, 8 aa, Ferroplasma acidarmanus
QMIGRAGR

SEQ ID NO: 49 - protein, 9 aa, Ferroplasma acidarmanus
QMIGRAGRP

SEQ ID NO: 50 - protein, 8 aa, Methanocaldococcus fervens
QCIGRAGR

SEQ ID NO: 51 - protein, 9 aa, Methanocaldococcus fervens
QCIGRAGRP

SEQ ID NO: 52 - protein, 8 aa, Methanocaldococcus jannaschii
QCIGRAGR

SEQ ID NO: 53 - protein, 9 aa, Methanocaldococcus jannaschii
QCIGRAGRP

SEQ ID NO: 54 - protein, 8 aa, Methanocaldococcus infernus
QCIGRAGR

SEQ ID NO: 55 - protein, 9 aa, Methanocaldococcus infernus
QCIGRAGRP

SEQ ID NO: 56 - protein, 8 aa, Methanospirillum hungatei
QMAGRAGR

SEQ ID NO: 57 - protein, 9 aa, Methanospirillum hungatei
QMAGRAGRP

SEQ ID NO: 58 - protein, 8 aa, Archaeoglobus fulgidus
QMAGRAGR

SEQ ID NO: 59 - protein, 9 aa, Archaeoglobus fulgidus
QMAGRAGRP

SEQ ID NO: 60 - protein, 8 aa, Haloterrigena turkmenica
QMAGRAGR

SEQ ID NO: 61 - protein, 9 aa, Haloterrigena turkmenica
QMAGRAGRP

SEQ ID NO: 62 - protein, 8 aa, Haladaptatus paucihalophilus
QMFGRAGR

SEQ ID NO: 63 - protein, 9 aa, Haladaptatus paucihalophilus
QMFGRAGRP

SEQ ID NO: 64 - protein, 8 aa, Halobacterium sp.
QMFGRAGR

SEQ ID NO: 65 - protein, 9 aa, Halobacterium sp.
QMFGRAGRP

SEQ ID NO: 66 - protein, 8 aa, Artificial Sequence
  source: /note="Description of Artificial Sequence: Synthetic peptide"
  VARIANT (2)..(2): /replace="Met" or "Leu"
  MOD_RES (3)..(3): Any amino acid
  source: /note="See specification as filed for detailed description of substitutions and preferred embodiments"
  misc_feature (1)..(8): /note="Variant residues given in the sequence have no preference with respect to those in the annotations for variant positions"
QCXGRAGR

SEQ ID NO: 67 - DNA, 87 bp, Artificial Sequence
  source: /note="Description of Artificial Sequence: Synthetic oligonucleotide"
  modified_base (10)..(10): abasic nucleotide
aaaccttccncccgtaccgtgccgtaccgttccgttccgtaccgtatttttttttctcactatcgcattctcatgcaggtcgtagcc

SEQ ID NO: 68 - DNA, 45 bp, Artificial Sequence
  source: /note="Description of Artificial Sequence: Synthetic oligonucleotide"
cctgcatgagaatgcgatagtgagatttttttttttttttttttt

SEQ ID NO: 69 - DNA, 102 bp, Artificial Sequence
  source: /note="Description of Artificial Sequence: Synthetic polynucleotide"
  modified_base (19)..(20): abasic nucleotide
ctcacctatccttccactnnccccctttgggtttaaattttttcagatctcactatctttttaaagttttctcactatcgcattctcatgcaggtcgtagcc

SEQ ID NO: 70 - DNA, 91 bp, Artificial Sequence
  source: /note="Description of Artificial Sequence: Synthetic oligonucleotide"
  modified_base (19)..(20): abasic nucleotide
catcatcatcatcatcatnnccccctaaacaagaataccacgactagcatttttcagatctcactatcgcattctcatgcaggtcgtagcc

SEQ ID NO: 71 - DNA, 91 bp, Artificial Sequence; identical to SEQ ID NO: 70
  source: /note="Description of Artificial Sequence: Synthetic oligonucleotide"
  modified_base (19)..(20): abasic nucleotide

SEQ ID NO: 72 - DNA, 87 bp, Artificial Sequence; identical to SEQ ID NO: 67
  source: /note="Description of Artificial Sequence: Synthetic oligonucleotide"
  modified_base (10)..(10): abasic nucleotide

SEQ ID NO: 73 - DNA, 60 bp, Artificial Sequence
  source: /note="Description of Artificial Sequence: Synthetic oligonucleotide"
aaaaaaaatacggtacggaacggaacggtacggcacggtacgggtttttttttttttttt

SEQ ID NO: 74 - DNA, 14 bp, Artificial Sequence
  source: /note="Description of Artificial Sequence: Synthetic oligonucleotide"
atcatcatcatcat

SEQ ID NO: 75 - protein, 9 aa, Unknown
  source: /note="Description of Unknown: 'SF2' family motif sequence"
GFCCPQSIQ

SEQ ID NO: 76 - protein, 8 aa, Unknown
  source: /note="Description of Unknown: 'SF2' family motif sequence"
  MOD_RES (2)..(3): Any amino acid
  MOD_RES (5)..(5): Any amino acid
AXXGXGKT

SEQ ID NO: 77 - protein, 6 aa, Unknown
  source: /note="Description of Unknown: 'SF2' family motif sequence"
PTRELA

SEQ ID NO: 78 - protein, 4 aa, Unknown
  source: /note="Description of Unknown: 'SF2' family motif sequence"
TPGR

SEQ ID NO: 79 - protein, 6 aa, Unknown
  source: /note="Description of Unknown: 'SF2' family motif sequence"
VLDEAD

SEQ ID NO: 80 - protein, 4 aa, Unknown
  source: /note="Description of Unknown: 'SF2' family motif sequence"
FVNT

SEQ ID NO: 81 - protein, 8 aa, Unknown
  source: /note="Description of Unknown: 'SF2' family motif sequence"
  MOD_RES (6)..(7): Any amino acid
HRIGRXXR

SEQ ID NO: 82 - DNA, 18 bp, Artificial Sequence
  source: /note="Description of Artificial Sequence: Synthetic primer"
tctcgtcgctcatcaact

SEQ ID NO: 83 - DNA, 18 bp, Artificial Sequence
  source: /note="Description of Artificial Sequence: Synthetic primer"
gagtcgaggtcatatcgt

SEQ ID NO: 84 - DNA, 18 bp, Artificial Sequence
  source: /note="Description of Artificial Sequence: Synthetic primer"
gtctgcctatagtgagtc

SEQ ID NO: 85 - DNA, 65 bp, Artificial Sequence
  source: /note="Description of Artificial Sequence: Synthetic primer"
  modified_base (22)..(23): abasic nucleotide
tttttttttttttttccttccnnttttcttcttcttcaagaagaagatctcgtcgctcatcaact

SEQ ID NO: 86 - DNA, 65 bp, Artificial Sequence
  source: /note="Description of Artificial Sequence: Synthetic primer"
  modified_base (22)..(23): abasic nucleotide
tttttttttttttttccttccnnttttttaattaattttgttgttgtgagtcgaggtcatatcgt

SEQ ID NO: 87 - DNA, 41 bp, Artificial Sequence
  source: /note="Description of Artificial Sequence: Synthetic primer"
  source: /note="Description of Combined DNA/RNA Molecule: Synthetic primer"
  modified_base (9)..(9): deoxyuracil
  modified_base (19)..(19): deoxyuracil
  modified_base (27)..(27): deoxyuracil
  modified_base (36)..(36): deoxyuracil
atacggcgnccaccgaccncagcgtcngcctatagngagtc

SEQ ID NO: 88 - DNA, 29 bp, Artificial Sequence
  source: /note="Description of Artificial Sequence: Synthetic oligonucleotide"
accgacactgcgtctgcctatagtgagtc

SEQ ID NO: 89 - DNA, 20 bp, Artificial Sequence
  source: /note="Description of Artificial Sequence: Synthetic oligonucleotide"
ttaattaattttgttgttgt

SEQ ID NO: 90 - DNA, 20 bp, Artificial Sequence
  source: /note="Description of Artificial Sequence: Synthetic oligonucleotide"
cttcttcttcaagaagaaga